European Patent Specification EP 3 700 904 B1, published July 19, 2023. Title: 4H-Pyrrolo[3,2-c]pyridin-4-one Derivatives. Applicant: Bayer Pharma AG Bayer AG The Broad Institute, Inc. Dana-Farber Cancer Institute, Inc. The sequence listing filed with the application follows.

SEQUENCE LISTING (5 sequences)

SEQ ID NO: 1 - protein, 788 aa, Artificial Sequence
  Modified Sequence
MSPILGYWKIKGLVQPTRLLLEYLEEKYEEHLYERDEGDKWRNKKFELGLEFPNLPYYIDGDVKLTQSMAIIRYIADKHNMLGGCPKERAEISMLEGAVLDIRYGVSRIAYSKDFETLKVDFLSKLPEMLKMFEDRLCHKTYLNGDHVTHPDFMLYDALDVVLYMDPMCLDAFPKLVCFKKRIEAIPQIDKYLKSSKYIAWPLQGWQATFGGGDHPPKSDPITSLYKKAGSDYDIPTTTENLYFQGRRRHIVRKRTLRRLLQERELVEPLTPSGEAPNQALLRILKETEFKKIKVLGSGAFGTVYKGLWIPEGEKVKIPVAIKELREATSPKANKEILDEAYVMASVDNPHVCRLLGICLTSTVQLITQLMPFGCLLDYVREHKDNIGSQYLLNWCVQIAKGMNYLEDRRLVHRDLAARNVLVKTPQHVKITDFGLAKLLGAEEKEYHAEGGKVPIKWMALESILHRIYTHQSDVWSYGVTVWELMTFGSKPYDGIPASEISSILEKGERLPQPPICTIDVYMIMVKCWMIDADSRPKFRELIIEFSKMARDPQRYLVIQGDERMHLPSPTDSNFYRALMDEEDMDDVVDADEYLIPQQGFFSSPSTSRTPLLSSLSATSNNSTVACIDRNGLQSCPIKEDSFLQRYSSDPTGALTEDSIDDTFLPVPEYINQSVPKRPAGSVQNPVYHNQPLNPAPSRDPHYQDPHSTAVGNPEYLNTVQPTCVNSTFDSPAHWAQKGSHQISLDNPDYQQDFFPKEAKPNGIFKGSTAENAEYLRVAPQSSEFIGA

SEQ ID NO: 2 - protein, 791 aa, Artificial Sequence
  Modified Sequence
MSPILGYWKIKGLVQPTRLLLEYLEEKYEEHLYERDEGDKWRNKKFELGLEFPNLPYYIDGDVKLTQSMAIIRYIADKHNMLGGCPKERAEISMLEGAVLDIRYGVSRIAYSKDFETLKVDFLSKLPEMLKMFEDRLCHKTYLNGDHVTHPDFMLYDALDVVLYMDPMCLDAFPKLVCFKKRIEAIPQIDKYLKSSKYIAWPLQGWQATFGGGDHPPKSDPITSLYKKAGSDYDIPTTTENLYFQGRRRHIVRKRTLRRLLQERELVEPLTPSGEAPNQALLRILKETEFKKIKVLGSGAFGTVYKGLWIPEGEKVKIPVAIKELREATSPKANKEILDEAYVMASVDASVNPHVCRLLGICLTSTVQLITQLMPFGCLLDYVREHKDNIGSQYLLNWCVQIAKGMNYLEDRRLVHRDLAARNVLVKTPQHVKITDFGLAKLLGAEEKEYHAEGGKVPIKWMALESILHRIYTHQSDVWSYGVTVWELMTFGSKPYDGIPASEISSILEKGERLPQPPICTIDVYMIMVKCWMIDADSRPKFRELIIEFSKMARDPQRYLVIQGDERMHLPSPTDSNFYRALMDEEDMDDVVDADEYLIPQQGFFSSPSTSRTPLLSSLSATSNNSTVACIDRNGLQSCPIKEDSFLQRYSSDPTGALTEDSIDDTFLPVPEYINQSVPKRPAGSVQNPVYHNQPLNPAPSRDPHYQDPHSTAVGNPEYLNTVQPTCVNSTFDSPAHWAQKGSHQISLDNPDYQQDFFPKEAKPNGIFKGSTAENAEYLRVAPQSSEFIGA

SEQ ID NO: 3 - protein, 791 aa, Artificial Sequence
  Modified Sequence
MSPILGYWKIKGLVQPTRLLLEYLEEKYEEHLYERDEGDKWRNKKFELGLEFPNLPYYIDGDVKLTQSMAIIRYIADKHNMLGGCPKERAEISMLEGAVLDIRYGVSRIAYSKDFETLKVDFLSKLPEMLKMFEDRLCHKTYLNGDHVTHPDFMLYDALDVVLYMDPMCLDAFPKLVCFKKRIEAIPQIDKYLKSSKYIAWPLQGWQATFGGGDHPPKSDPITSLYKKAGSDYDIPTTTENLYFQGRRRHIVRKRTLRRLLQERELVEPLTPSGEAPNQALLRILKETEFKKIKVLGSGAFGTVYKGLWIPEGEKVKIPVAIKELREATSPKANKEILDEAYVMASVDSVDNPHVCRLLGICLTSTVQLITQLMPFGCLLDYVREHKDNIGSQYLLNWCVQIAKGMNYLEDRRLVHRDLAARNVLVKTPQHVKITDFGLAKLLGAEEKEYHAEGGKVPIKWMALESILHRIYTHQSDVWSYGVTVWELMTFGSKPYDGIPASEISSILEKGERLPQPPICTIDVYMIMVKCWMIDADSRPKFRELIIEFSKMARDPQRYLVIQGDERMHLPSPTDSNFYRALMDEEDMDDVVDADEYLIPQQGFFSSPSTSRTPLLSSLSATSNNSTVACIDRNGLQSCPIKEDSFLQRYSSDPTGALTEDSIDDTFLPVPEYINQSVPKRPAGSVQNPVYHNQPLNPAPSRDPHYQDPHSTAVGNPEYLNTVQPTCVNSTFDSPAHWAQKGSHQISLDNPDYQQDFFPKEAKPNGIFKGSTAENAEYLRVAPQSSEFIGA

SEQ ID NO: 4 - protein, 14 aa, Artificial Sequence
  MOD_RES 1: Biotin-Ahx
  Modified Sequence
  MOD_RES 14: AMIDATION
AEEEEYFELVAKKK

SEQ ID NO: 5 - protein, 12 aa, Artificial Sequence
  MOD_RES 1: Biotin-Ahx
  Modified Sequence
  MOD_RES 12: AMIDATION
VLLPKKSFAEPG